European Patent Application EP 4 667 496 A2, published December 24, 2025. Title: FACTOR X BINDERS ENHANCING FX ACTIVATION. Applicant: Novo Nordisk A/S. Application EP PCT/EP2018/081296, filed November 15, 2018. The sequence listing filed with the application follows.

SEQUENCE LISTING (57 sequences)

SEQ ID NO: 1 - protein, 415 aa, Homo sapiens
YNSGKLEEFVQGNLERECMEEKCSFEEAREVFENTERTTEFWKQYVDGDQCESNPCLNGGSCKDDINSYECWCPFGFEGKNCELDVTCNIKNGRCEQFCKNSADNKVVCSCTEGYRLAENQKSCEPAVPFPCGRVSVSQTSKLTRAEAVFPDVDYVNSTEAETILDNITQSTQSFNDFTRVVGGEDAKPGQFPWQVVLNGKVDAFCGGSIVNEKWIVTAAHCVETGVKITVVAGEHNIEETEHTEQKRNVIRIIPHHNYNAAINKYNHDIALLELDEPLVLNSYVTPICIADKEYTNIFLKFGSGYVSGWGRVFHKGRSALVLQYLRVPLVDRATCLRSTKFTIYNNMFCAGFHEGGRDSCQGDSGGPHVTEVEGTSFLTGIISWGEECAMKGKYGIYTKVSRYVNWIKEKTKLT

SEQ ID NO: 2 - protein, 448 aa, Homo sapiens [sequence omitted]

SEQ ID NO: 3 - skipped

SEQ ID NO: 4 - protein, 117 aa, Homo sapiens
  REGION 1..117: note = Antibody heavy chain variable domain
QSVEESGGRLVTPGTPLTLTCTVSGFSLSSYAMSWVRQAPGKGLEWIGIISTSGSTFYATWAKGRFTISKTSTTVDLKIISPTIEDTATYFCARDMWAGSRYDFNIWGPGTLVTVSS

SEQ ID NO: 5 - protein, 113 aa, synthetic construct
  REGION 1..113: note = Antibody light chain variable domain
ADIVMTQTPASVEAAVGGTVTIKCQASQSISSYLAWYQQKPGQRPKLLIYRASTLESGVPSRFKGSGSGTQFTLTISDLECADAATYYCQTYYYSGGGSYASAFGGGTEVVVK

SEQ ID NO: 6 - protein, 117 aa, synthetic construct
  REGION 1..117: note = Antibody heavy chain variable domain
EVQLVESGGGQVKPGGSLRLSCAASGFTFSTSSIYWVRQAPGKGLEWVSSISSGSSYIFYADSVKGRFTISRDNAKNSLFLQMNSLRAEDTAVYYCVSGYSRLLDYWGQGTLVTVSS

SEQ ID NO: 7 - protein, 112 aa, synthetic construct
  REGION 1..112: note = Antibody light chain variable domain
DVVMTQSPLSLPVTLGQPASISCRSSQSLVYSDGNTYLNWFQQRPGQSPRRLIYKVSNRDSGVPDRFSGSGSGTDFTLKISRVEAEDVGFYYCMQGTHWPLTFGGGTKVEIK

SEQ ID NO: 8 - protein, 120 aa, synthetic construct
  REGION 1..120: note = Single variable domain antibody
EVQLVESGGGVVQPGGSLRLSCAASGRTFSTYAMGWFRQAPGKEREFVAAISWSGSRTYYADSVKGRFTISRDNSKNTVYLQMNSLRPEDTALYYCAADATPANGELDYWGQGTLVTVSS

SEQ ID NO: 9 - protein, 120 aa, synthetic construct
  REGION 1..120: note = Single variable domain antibody
EVQLVESGGGVVQPGGSLRLSCAASGRTFSTYAMGWFRQAPGKEREFVAAISRRGGRTYYADSVKGRFTISRDNSKNTVYLQMNSLRPEDTALYYCAADATARDGLLDYWGQGTLVTVSS

SEQ ID NO: 10 - protein, 120 aa, synthetic construct
  REGION 1..120: note = Single variable domain antibody
EVQLVESGGGVVQPGGSLRLSCVASGRTFSRYAMGWFRQAPGKEREFVAAISRRGGSTNYADSVKGRFTISRDNSKNTVYLQMNSLRPEDTALYYCAADYSSGDGYLDYWGQGTLVTVSS

SEQ ID NO: 11 - protein, 120 aa, synthetic construct
  REGION 1..120: note = Single variable domain antibody
EVQLVESGGGVVQPGGSLRLSCAASGGTLSRYAMGWFRQAPGKEREFVAAITRRGSRTYYADSVKGRFTISRDNSKNTVYLQMNSLRPEDTALYYCAADLAPGDYALDYWGQGTLVTVSS

SEQ ID NO: 12 - protein, 121 aa, synthetic construct
  REGION 1..121: note = Single variable domain antibody
EVQLVESGGGLVQPGGSLRLSCAASGFTFSNYEMSWVRQAPGKGLEWVSDIGSGGGVSTYYADSVKGRFTISRDNAKNTLYLQMNSLKPEDTAMYYCARGWTYGSDGMDYWGKGTLVTVSS

SEQ ID NO: 13 - protein, 12 aa, Human
SVAQATSSSGEA

SEQ ID NO: 14 - protein, 12 aa, Human
VAQATSSSGEAP

SEQ ID NO: 15 - protein, 12 aa, Human
AQATSSSGEAPD

SEQ ID NO: 16 - protein, 12 aa, Human
QATSSSGEAPDS

SEQ ID NO: 17 - protein, 12 aa, Human
ATSSSGEAPDSI

SEQ ID NO: 18 - protein, 12 aa, Human
TSSSGEAPDSIT

SEQ ID NO: 19 - protein, 12 aa, Human
SSSGEAPDSITW

SEQ ID NO: 20 - protein, 12 aa, Human
SSGEAPDSITWK

SEQ ID NO: 21 - protein, 12 aa, Human
SGEAPDSITWKP

SEQ ID NO: 22 - protein, 12 aa, Human
GEAPDSITWKPY

SEQ ID NO: 23 - protein, 12 aa, Human
EAPDSITWKPYD

SEQ ID NO: 24 - protein, 12 aa, Human
APDSITWKPYDA

SEQ ID NO: 25 - protein, 12 aa, Human
PDSITWKPYDAA

SEQ ID NO: 26 - protein, 12 aa, Human
DSITWKPYDAAD

SEQ ID NO: 27 - protein, 12 aa, Human
SITWKPYDAADL

SEQ ID NO: 28 - protein, 12 aa, Human
ITWKPYDAADLD

SEQ ID NO: 29 - protein, 12 aa, Human
TWKPYDAADLDP

SEQ ID NO: 30 - protein, 12 aa, Human
WKPYDAADLDPT

SEQ ID NO: 31 - protein, 12 aa, Human
KPYDAADLDPTE

SEQ ID NO: 32 - protein, 12 aa, Human
PYDAADLDPTEN

SEQ ID NO: 33 - protein, 12 aa, Human
YDAADLDPTENP

SEQ ID NO: 34 - protein, 12 aa, Human
DAADLDPTENPF

SEQ ID NO: 35 - protein, 12 aa, Human
AADLDPTENPFD

SEQ ID NO: 36 - protein, 12 aa, Human
ADLDPTENPFDL

SEQ ID NO: 37 - protein, 12 aa, Human
DLDPTENPFDLL

SEQ ID NO: 38 - protein, 12 aa, Human
LDPTENPFDLLD

SEQ ID NO: 39 - protein, 12 aa, Human
DPTENPFDLLDF

SEQ ID NO: 40 - protein, 12 aa, Human
PTENPFDLLDFN

SEQ ID NO: 41 - protein, 12 aa, Human
TENPFDLLDFNQ

SEQ ID NO: 42 - protein, 12 aa, Human
ENPFDLLDFNQT

SEQ ID NO: 43 - protein, 12 aa, Human
NPFDLLDFNQTQ

SEQ ID NO: 44 - protein, 12 aa, Human
PFDLLDFNQTQP

SEQ ID NO: 45 - protein, 12 aa, Human
FDLLDFNQTQPE

SEQ ID NO: 46 - protein, 12 aa, Human
DLLDFNQTQPER

SEQ ID NO: 47 - protein, 12 aa, Human
LLDFNQTQPERG

SEQ ID NO: 48 - protein, 12 aa, Human
LDFNQTQPERGD

SEQ ID NO: 49 - protein, 12 aa, Human
DFNQTQPERGDN

SEQ ID NO: 50 - protein, 12 aa, Human
FNQTQPERGDNN

SEQ ID NO: 51 - protein, 12 aa, Human
NQTQPERGDNNL

SEQ ID NO: 52 - protein, 12 aa, Human
QTQPERGDNNLT

SEQ ID NO: 53 - protein, 12 aa, Human
TQPERGDNNLTR

SEQ ID NO: 54 - protein, 120 aa, synthetic construct
  REGION 1..120: note = Single variable domain antibody
EVQLVESGGGVVQPGGSLRLSCAASGRTFSTYSMGWFRQAPGKEREFVAAITRRGSRTYYADSVKGRFTISRDNSKNTVYLQMNSLRPEDTALYYCAADRRPADSYLDYWGQGTLVTVSS

SEQ ID NO: 55 - protein, 121 aa, synthetic construct
  REGION 1..121: note = Single variable domain antibody
EVQLVESGGGVVQPGGSLRLSCAASGFTFSDYAMSWVRQAPGKGLEWVSGITSGGGRTYYADSVKGRFTISRDNSKNTLYLQMNSLRPEDTALYYCAAVRTLGLRGSYDYWGQGTLVTVSS

SEQ ID NO: 56 - protein, 120 aa, synthetic construct
  REGION 1..120: note = Single variable domain antibody
EVQLVESGGGVVQPGGSLRLSCAASGFTFSDYAMSWVRQAPGKGLEWVSGITGGGRTYYADSVKGRFTISRDNSKNTLYLQMNSLRPEDTALYYCAAAILTRTRRTYDYWGQGTLVTVSS

SEQ ID NO: 57 - protein, 121 aa, synthetic construct
  REGION 1..121: note = Single variable domain antibody
EVQLVESGGGVVQPGGSLRLSCVASGFTFSDYAMSWVRQAPGKGLEWVSGITSGSGRTYYADSVKGRFTISRDNSKNTVYLQMNSLRPEDTALYYCAAAILRGYRKTYDYWGQGTLVTVSS